European Patent Application EP 4 112 079 A1, published January 4, 2023. Title: Dosage Regimen for MAdCAM Antagonists. Applicant: Pfizer Inc. The sequence listing filed with the application follows.

SEQUENCE LISTING (38 sequences)

SEQ ID NO: 1 - protein, 219 aa, Artificial Sequence
  Synthetic Construct
DIVMTQTPLSLSVTPGQPASISCKSSQSLLHTDGTTYLYWYLQKPGQPPQLLIYEVSNRFSGVPDRFSGSGSGTDFTLKISRVEAEDVGIYYCMQNIQLPWTFGQGTKVEIKRTVAAPSVFIFPPSDEQLKSGTASVVCLLNNFYPREAKVQWKVDNALQSGNSQESVTEQDSKDSTYSLSSTLTLSKADYEKHKVYACEVTHQGLSSPVTKSFNRGEC

SEQ ID NO: 2 - protein, 450 aa, Artificial Sequence
  Synthetic Construct
QVQLVQSGAEVKKPGASVKVSCKASGYTFTSYGINWVRQAPGQGLEWMGWISVYSGNTNYAQKVQGRVTMTADTSTSTAYMDLRSLRSDDTAVYYCAREGSSSSGDYYYGMDVWGQGTTVTVSSASTKGPSVFPLAPCSRSTSESTAALGCLVKDYFPEPVTVSWNSGALTSGVHTFPAVLQSSGLYSLSSVVTVPSSNFGTQTYTCNVDHKPSNTKVDKTVERKCCVECPPCPAPPVAGPSVFLFPPKPKDTLMISRTPEVTCVVVDVSHEDPEVQFNWYVDGVEVHNAKTKPREEQFNSTFRVVSVLTVVHQDWLNGKEYKCKVSNKGLPAPIEKTISKTKGQPREPQVYTLPPSREEMTKNQVSLTCLVKGFYPSDIAVEWESNGQPENNYKTTPPMLDSDGSFFLYSKLTVDKSRWQQGNVFSCSVMHEALHNHYTQKSLSLSPGK

SEQ ID NO: 3 - protein, 112 aa, Artificial Sequence
  Synthetic Construct
DIVMTQTPLSLSVTPGQPASISCKSSQSLLHTDGTTYLYWYLQKPGQPPQLLIYEVSNRFSGVPDRFSGSGSGTDFTLKISRVEAEDVGIYYCMQNIQLPWTFGQGTKVEIK

SEQ ID NO: 4 - protein, 124 aa, Artificial Sequence
  Synthetic Construct
QVQLVQSGAEVKKPGASVKVSCKASGYTFTSYGINWVRQAPGQGLEWMGWISVYSGNTNYAQKVQGRVTMTADTSTSTAYMDLRSLRSDDTAVYYCAREGSSSSGDYYYGMDVWGQGTTVTVSS

SEQ ID NO: 5 - protein, 107 aa, Artificial Sequence [sequence omitted]

SEQ ID NO: 6 - protein, 101 aa, Artificial Sequence
  Synthetic Construct
ASTKGPSVFPLAPCSRSTSESTAALGCLVKDYFPEPVTVSWNSGALTSGVHTFPAVLQSSGLYSLSSVVTVPSSNFGTQTYTCNVDHKPSNTKVDKTVERK

SEQ ID NO: 7 - protein, 9 aa, Artificial Sequence
  Synthetic Construct
CCVECPPCP

SEQ ID NO: 8 - protein, 109 aa, Artificial Sequence
  Synthetic Construct
APPVAGPSVFLFPPKPKDTLMISRTPEVTCVVVDVSHEDPEVQFNWYVDGVEVHNAKTKPREEQFNSTFRVVSVLTVVHQDWLNGKEYKCKVSNKGLPAPIEKTISKTK

SEQ ID NO: 9 - protein, 107 aa, Artificial Sequence
  Synthetic Construct
GQPREPQVYTLPPSREEMTKNQVSLTCLVKGFYPSDIAVEWESNGQPENNYKTTPPMLDSDGSFFLYSKLTVDKSRWQQGNVFSCSVMHEALHNHYTQKSLSLSPGK

SEQ ID NO: 10 - protein, 326 aa, Artificial Sequence
  Synthetic Construct
ASTKGPSVFPLAPCSRSTSESTAALGCLVKDYFPEPVTVSWNSGALTSGVHTFPAVLQSSGLYSLSSVVTVPSSNFGTQTYTCNVDHKPSNTKVDKTVERKCCVECPPCPAPPVAGPSVFLFPPKPKDTLMISRTPEVTCVVVDVSHEDPEVQFNWYVDGVEVHNAKTKPREEQFNSTFRVVSVLTVVHQDWLNGKEYKCKVSNKGLPAPIEKTISKTKGQPREPQVYTLPPSREEMTKNQVSLTCLVKGFYPSDIAVEWESNGQPENNYKTTPPMLDSDGSFFLYSKLTVDKSRWQQGNVFSCSVMHEALHNHYTQKSLSLSPGK

SEQ ID NO: 11 - protein, 16 aa, Artificial Sequence
  Synthetic Construct
KSSQSLLHTDGTTYLY

SEQ ID NO: 12 - protein, 7 aa, Artificial Sequence
  Synthetic Construct
EVSNRFS

SEQ ID NO: 13 - protein, 9 aa, Artificial Sequence
  Synthetic Construct
MQNIQLPWT

SEQ ID NO: 14 - protein, 5 aa, Artificial Sequence
  Synthetic Construct
SYGIN

SEQ ID NO: 15 - protein, 17 aa, Artificial Sequence
  Synthetic Construct
WISVYSGNTNYAQKVQG

SEQ ID NO: 16 - protein, 15 aa, Artificial Sequence
  Synthetic Construct
EGSSSSGDYYYGMDV

SEQ ID NO: 17 - protein, 218 aa, Artificial Sequence
  Synthetic Construct
DIVMTQSPLSLPVTPGEPASISCRSSQSLLQSNGYNYLDWYLQKPGQSPQLLIYLGSNRASGVPDRFSGSGSGTDFTLKISRVEAEDVGVYYCMQALQTITFGQGTRLEIKRTVAAPSVFIFPPSDEQLKSGTASVVCLLNNFYPREAKVQWKVDNALQSGNSQESVTEQDSKDSTYSLSSTLTLSKADYEKHKVYACEVTHQGLSSPVTKSFNRGEC

SEQ ID NO: 18 - protein, 444 aa, Artificial Sequence
  Synthetic Construct
EVQLVESGGGLVKPGGSLRLSCVASGFTFTNAWMIWVRQAPGKGLEWVGRIKRKTDGGTTDYAAPVKGRFTISRDDSKNTLYLQMNSLKTEDTAVYYCTTGGVAEDYWGQGTLVTVSSASTKGPSVFPLAPCSRSTSESTAALGCLVKDYFPEPVTVSWNSGALTSGVHTFPAVLQSSGLYSLSSVVTVPSSNFGTQTYTCNVDHKPSNTKVDKTVERKCCVECPPCPAPPVAGPSVFLFPPKPKDTLMISRTPEVTCVVVDVSHEDPEVQFNWYVDGVEVHNAKTKPREEQFNSTFRVVSVLTVVHQDWLNGKEYKCKVSNKGLPAPIEKTISKTKGQPREPQVYTLPPSREEMTKNQVSLTCLVKGFYPSDIAVEWESNGQPENNYKTTPPMLDSDGSFFLYSKLTVDKSRWQQGNVFSCSVMHEALHNHYTQKSLSLSPGK

SEQ ID NO: 19 - protein, 218 aa, Artificial Sequence
  Synthetic Construct
DIVMTQSPLSLPVTPGEPASISCRSSQSLLQSNGFNYLDWYLQKPGQSPQLLIYLGSNRASGVPDRFSGSGSGTDFTLKISRVEAEDVGVYYCMQALQTITFGQGTRLEIKRTVAAPSVFIFPPSDEQLKSGTASVVCLLNNFYPREAKVQWKVDNALQSGNSQESVTEQDSKDSTYSLSSTLTLSKADYEKHKVYACEVTHQGLSSPVTKSFNRGEC

SEQ ID NO: 20 - protein, 444 aa, Artificial Sequence
  Synthetic Construct
EVQLVESGGGLVKPGGSLRLSCVVSGFTFTNAWMIWVRQAPGKGLEWVGRIKRKTDGGTTDYAAPVKGRFTISRDDSKNTLYLQMNSLKTEDTAVYYCTTGGVAEDYWGQGTLVTVSSASTKGPSVFPLAPCSRSTSESTAALGCLVKDYFPEPVTVSWNSGALTSGVHTFPAVLQSSGLYSLSSVVTVPSSNFGTQTYTCNVDHKPSNTKVDKTVERKCCVECPPCPAPPVAGPSVFLFPPKPKDTLMISRTPEVTCVVVDVSHEDPEVQFNWYVDGVEVHNAKTKPREEQFNSTFRVVSVLTVVHQDWLNGKEYKCKVSNKGLPAPIEKTISKTKGQPREPQVYTLPPSREEMTKNQVSLTCLVKGFYPSDIAVEWESNGQPENNYKTTPPMLDSDGSFFLYSKLTVDKSRWQQGNVFSCSVMHEALHNHYTQKSLSLSPGK

SEQ ID NO: 21 - protein, 214 aa, Artificial Sequence
  Synthetic Construct
DIQMTQSPSSLSASVGDRVTITCRASRSISSYLNWYQQKPGKAPKVLIFFVSSLQSGVPSRFSGSGSGTDFTLTISSLQPEDFATYYCQQNYIPPITFGQGTRLEIRRTVAAPSVFIFPPSDEQLKSGTASVVCLLNNFYPREAKVQWKVDNALQSGNSQESVTEQDSKDSTYSLSSTLTLSKADYEKHKVYACEVTHQGLSSPVTKSFNRGEC

SEQ ID NO: 22 - protein, 448 aa, Artificial Sequence
  Synthetic Construct
EVQLLESGGGLVQPGGSLRLSCAASGLTFNNSAMTWVRQAPGKGLEWVSTTSGSGGTTYYADSVKGRFTISRDSPKNTLYLQMNSLRAEDTAVYYCAARGYSYGTTPYEYWGQGTLVTVSSASTKGPSVFPLAPCSRSTSESTAALGCLVKDYFPEPVTVSWNSGALTSGVHTFPAVLQSSGLYSLSSVVTVPSSSLGTKTYTCNVDHKPSNTKVDKRVESKYGPPCPSCPAPEFLGGPSVFLFPPKPKDTLMISRTPEVTCVVVDVSQEDPEVQFNWYVDGVEVHNAKTKPREEQFNSTYRVVSVLTVLHQDWLNGKEYKCKVSNKGLPSSIEKTISKAKGQPREPQVYTLPPSQEEMTKNQVSLTCLVKGFYPSDIAVEWESNGQPENNYKTTPPVLDSDGSFFLYSRLTVDKSRWQEGNVFSCSVMHEALHNHYTQKSLSLSLGK

SEQ ID NO: 23 - protein, 214 aa, Artificial Sequence
  Synthetic Construct
EIVLTQSPDFQSVTPKEKVTITCRASQRIGSSLHWYQQKPDQSPKLLIKYASQSFSGVPSRFSGSGSGTNFTLTINGLEAEDAATYYCHQSGRLPLTFGGGTKVEIKRTVAAPSVFIFPPSDEQLKSGTASVVCLLNNFYPREAKVQWKVDNALQSGNSQESVTEQDSKDSTYSLSSTLTLSKADYEKHKVYACEVTHQGLSSPVTKSFNRGEC

SEQ ID NO: 24 - protein, 446 aa, Artificial Sequence
  Synthetic Construct
QVQLVESGGGVVQPGRSLRLSCAASGHTFSSDGMHWVRQAPGKGLEWVAIIWYDGSNKYYADSVKGRFTISRDNSKNTLYLQMNSLRAEDTAVYYCARDPGYYYGMDVWGQGTTVTVSSASTKGPSVFPLAPCSRSTSESTAALGCLVKDYFPEPVTVSWNSGALTSGVHTFPAVLQSSGLYSLSSVVTVPSSSLGTKTYTCNVDHKPSNTKVDKRVESKYGPPCPSCPAPEFLGGPSVFLFPPKPKDTLMISRTPEVTCVVVDVSQEDPEVQFNWYVDGVEVHNAKTKPREEQFNSTYRVVSVLTVLHQDWLNGKEYKCKVSNKGLPSSIEKTISKAKGQPREPQVYTLPPSQEEMTKNQVSLTCLVKGFYPSDIAVEWESNGQPENNYKTAPPVLDSDGSFFLYSRLTVDKSRWQEGNVFSCSVMHEALHNHYTQKSLSLSLGK

SEQ ID NO: 25 - protein, 214 aa, Artificial Sequence
  Synthetic Construct
DIQMTQSPSSLSASVGDRVTITCRASQNISSYLNWFQQKPGKAPKLLIYAASGLKRGVPSRFSGSGSGTDFTLTIRTLQPDDFATYSCHQSYSLPFTFGPGTKVDIKRTVAAPSVFIFPPSDEQLKSGTASVVCLLNNFYPREAKVQWKVDNALQSGNSQESVTEQDSKDSTYSLSSTLTLSKADYEKHKVYACEVTHQGLSSPVTKSFNRGEC

SEQ ID NO: 26 - protein, 450 aa, Artificial Sequence
  Synthetic Construct
QVQLVESGGGVVQPGRSLRLSCAASGFTFSSYGMHWVRQAPGKGLEWVAVISNDGNNKYYADSVKGRFTISRDNSKNTLYLQMNSLSAEDTAVYYCARDSTAITYYYYGMDVWGQGTTVTVSSASTKGPSVFPLAPCSRSTSESTAALGCLVKDYFPEPVTVSWNSGALTSGVHTFPAVLQSSGLYSLSSVVTVPSSSLGTKTYTCNVDHKPSNTKVDKRVESKYGPPCPSCPAPEFLGGPSVFLFPPKPKDTLMISRTPEVTCVVVDVSQEDPEVQFNWYVDGVEVHNAKTKPREEQFNSTYRVVSVLTVLHQDWLNGKEYKCKVSNKGLPSSIEKTISKAKGQPREPQVYTLPPSQEEMTKNQVSLTCLVKGFYPSDIAVEWESNGQPENNYKTTPPVLDSDGSFFLYSRLTVDKSRWQEGNVFSCSVMHEALHNHYTQKSLSLSLGK

SEQ ID NO: 27 - protein, 221 aa, Artificial Sequence
  Synthetic Construct
DIVMTQSPDSLAVSLGERATINCKSSQSVLYSSNNKTYLAWYQQKPRQPPKLLIYWASIREYGVPDRFSGSGSGTDFTLTISSLQAEDVAVYFCQQYYSIPPLTFGGGTKVEIKRTVAAPSVFIFPPSDEQLKSGTASVVCLLNNFYPREAKVQWKVDNALQSGNSQESVTEQDSKDSTYSLSSTLTLSKADYEKHKVYACEVTHQGLSSPVTKSFNRGEC

SEQ ID NO: 28 - protein, 451 aa, Artificial Sequence
  Synthetic Construct
QVQLQESGPGLVKPSETLSLTCTVSGDSISSNYWSWIRQPAGKGLEWIGRIYTSGGTNSNPSLRGRVTILADTSKNQFSLKLSSVTAADTAVYYCARDRITIIRGLIPSFFDYWGQGTLVTVSSASTKGPSVFPLAPCSRSTSESTAALGCLVKDYFPEPVTVSWNSGALTSGVHTFPAVLQSSGLYSLSSVVTVPSSSLGTKTYTCNVDHKPSNTKVDKRVESKYGPPCPSCPAPEFLGGPSVFLFPPKPKDTLMISRTPEVTCVVVDVSQEDPEVQFNWYVDGVEVHNAKTKPREEQFNSTYRVVSVLTVLHQDWLNGKEYKCKVSNKGLPSSIEKTISKAKGQPREPQVYTLPPSQEEMTKNQVSLTCLVKGFYPSDIAVEWESNGQPENNYKTTPPVLDSDGSFFLYSRLTVDKSRWQEGNVFSCSVMHEALHNHYTQKSLSLSLGK

SEQ ID NO: 29 - protein, 216 aa, Artificial Sequence
  Synthetic Construct
DIQMTQSPSSLSASVGDRVTFTCRASQNITNYLNWYQQKPGKAPKLLIYAASSLPRGVPSRFRGSGSGTDFTLTISSLQPEDFATYYCQQSYSNPPECGFGQGTTLDIKRTVAAPSVFIFPPSDEQLKSGTASVVCLLNNFYPREAKVQWKVDNALQSGNSQESVTEQDSKDSTYSLSSTLTLSKADYEKHKVYACEVTHQGLSSPVTKSFNRGEC

SEQ ID NO: 30 - protein, 452 aa, Artificial Sequence
  Synthetic Construct
EVQLLESGGDLVQPGGSLRLSCAASGFTFRSYAMNWVRQAPGKGLEWVSVISGRGGTTYYADSVKGRFTISRDNSKNTLYLQMNSLRAEDAAVYYCAKIAVAGEGLYYYYGMDVWGQGTTVTVSSASTKGPSVFPLAPCSRSTSENTAALGCLVKDYFPEPVTVSWNSGALTSGVHTFPAVLQSSGLYSLSSVVTVPSSSLGTKTYTCNVDHKPSNTKVDKRVESKYGPPCPSCPAPEFLGGPSVFLFPPKPKDTLMISRTPEVTCVVVDVSQEDPEVQFNWYVDGVEVHNAKTKPREEQFNSTYRVVSVLTVLHQDWLNGKEYKCKVSNKGLPSSIEKTISKAKGQPREPQVYTLPPSQEEMTKNQVSLTCLVKGFYPSDIAVEWESNGQPENNYKTTPPVLDSDGSFFLYSRLTVDKSRWQEGNVFSCSVMHEALHNHYTQKSLSLSLGK

SEQ ID NO: 31 - protein, 219 aa, Artificial Sequence
  Synthetic Construct
DIVMTQTPLSLSVTPGQPASISCNSSQSLLLSDGKTYLNWYLQKPGQPPQLLIYEVSNRFSGVPDRFSGSGSGTDFTLKISRVEAEDVGVYSCMQSIQLMCSFGQGTKLEIKRTVAAPSVFIFPPSDEQLKSGTASVVCLLNNFYPREAKVQWKVDNALQSGNSQESVTEQDSKDSTYSLSSTLTLSKADYEKHKVYACEVTHQGLSSPVTKSFNRGEC

SEQ ID NO: 32 - protein, 453 aa, Artificial Sequence
  Synthetic Construct
EVQLVESGGGLVKPGGSLRLSCAASGFTFSSYSMNWVRQAPGKGLEWVSSISSSSSYIYYADSVKGRFTISRDNAKNSLYLQMNSLRAEDTAVYYCARDGYSSGWSYYYYYGMDVWGQGTTVTVSSASTKGPSVFPLAPCSRSTSESTAALGCLVKDYFPEPVTVSWNSGALTSGVHTFPAVLQSSGLYSLSSVVTVPSSSLGTKTYTCNVDHKPSNTKVDKRVESKYGPPCPSCPAPEFLGGPSVFLFPPKPKDTLMISRTPEVTCVVVDVSQEDPEVQFNWYVDGVEVHNAKTKPREEQFNSTYRVVSVLTVLHQDWLNGKEYKCKVSNKGLPSSIEKTISKAKGQPREPQVYTLPPSQEEMTKNQVSLTCLVKGFYPSDIAVEWESNGQPENNYKTTPPVLDSDGSFFLYSRLTVDKSRWQEGNVFSRSVMHEALHNHYTQKSLSLSLGK

SEQ ID NO: 33 - protein, 218 aa, Artificial Sequence
  Synthetic Construct
DIVMTQSPLSLPVTPGEPASISCRSSQSLLHGNGYNYLDWYLQKPGQSPQLLIYLGSNRASGVPDRFSGSGSGTDFTLKISRVEAEDVGVYYCMQALQTLTFGGGTKVEIKRTVAAPSVFIFPPSDEQLKSGTASVVCLLNNFYPREAKVQWKVDNALQSGNSQESVTEQDSKDSTYSLSSTLTLSKADYEKHKVYACEVTHQGLSSPVTKSFNRGEC

SEQ ID NO: 34 - protein, 452 aa, Artificial Sequence
  Synthetic Construct
QVQLQESGPGLVKPSETLSLTCTVSGSSISSYHWNWIRQPAGKGLEWIGRIYTSGSTNYNPSLKSRVTMSLDTSKNQFSLKLSSVTAADTAVYYCAREGVRYYYASGSYYYGLDVWGQGTTVTVSSASTKGPSVFPLAPCSRSTSESTAALGCLVKDYFPEPVTVSWNSGALTSGVHTFPAVLQSSGLYSLSSVVTVPSSNFGTQTYTCNVDHKPSNTKVDKTVERKCCVECPPCPAPPVAGPSVFLFPPKPKDTLMISRTPEVTCVVVDVSHEDPEVQFNWYVDGVEVHNAKTKPREEQFNSTFRVVSVLTVVHQDWLNGKEYKCKVSNKGLPAPIEKTISKTKGQPREPQVYTLPPSREEMTKNQVSLTCLVKGFYPSDIAVEWESNGQPENNYKTTPPMLDSDGSFFLYSKLTVDKSRWQQGNVFSCSVMHEALHNHYTQKSLSLSPGK

SEQ ID NO: 35 - protein, 219 aa, Artificial Sequence
  Synthetic Construct
DIVMTQTPLSLSVTPGQPASISCKSNQSLLYSDGKTYLFWYLQKPGQPPQLLIYEVSNRFSGVPDRFSGSGSGTDFTLKISRVEAEDVGVYYCMQSIQLPWTFGQGTKVEIKRTVAAPSVFIFPPSDEQLKSGTASVVCLLNNFYPREAKVQWKVDNALQSGNSQESVTEQDSKDSTYSLSSTLTLSKADYEKHKVYACEVTHQGLSSPVTKSFNRGEC

SEQ ID NO: 36 - protein, 450 aa, Artificial Sequence
  Synthetic Construct
QVQLVQSGAEVKKPGASVKVSCEASGYTFTSYGIDWVRQAPGQGLEWMGWISVYSGNTNYAQKLQGRVTMSTDTSTSTAYMELRSLRSDDTAVYYCAREGSSSSGDYYYGMDVWGQGTTVTVSSASTKGPSVFPLAPCSRSTSESTAALGCLVKDYFPEPVTVSWNSGALTSGVHTFPAVLQSSGLYSLSSVVTVPSSNFGTQTYTCNVDHKPSNTKVDKTVERKCCVECPPCPAPPVAGPSVFLFPPKPKDTLMISRTPEVTCVVVDVSHEDPEVQFNWYVDGVEVHNAKTKPREEQFNSTFRVVSVLTVVHQDWLNGKEYKCKVSNKGLPAPIEKTISKTKGQPREPQVYTLPPSREEMTKNQVSLTCLVKGFYPSDIAVEWESNGQPENNYKTTPPMLDSDGSFFLYSKLTVDKSRWQQGNVFSCSVMHEALHNHYTQKSLSLSPGK

SEQ ID NO: 37 - protein, 214 aa, Artificial Sequence
  Synthetic Construct
DIQMTQSPSSLSASVGDRVTITCQASQDISNYLNWYQQKPGKAPKLLIYDASNLETGVPSRFSGSGSGTDFTFTISSLQPEDIATYSCQHSDNLSITFGQGTRLEIKRTVAAPSVFIFPPSDEQLKSGTASVVCLLNNFYPREAKVQWKVDNALQSGNSQESVTEQDSKDSTYSLSSTLTLSKADYEKHKVYACEVTHQGLSSPVTKSFNRGEC

SEQ ID NO: 38 - protein, 443 aa, Artificial Sequence
  Synthetic Construct
QVQLVESGGGVVQPGRSLRLSCAASGFTFSSYGMHWVRQAPGKGLEWVAVIWYDGSNEYYADSVKGRFTISRDNSKNTLYLQMNSLRAEDTAVYYCARGAYHFAYWGQGTLVTVSSASTKGPSVFPLAPCSRSTSESTAALGCLVKDYFPEPVTVSWNSGALTSGVHTFPAVLQSSGLYSLSSVVTVPSSSLGTKTYTCNVDHKPSNTKVDKRVESKYGPPCPSCPAPEFLGGPSVFLFPPKPKDTLMISRTPEVTCVVVDVSQEDPEVQFNWYVDGVEVHNAKTKPREEQFNSTYRVVSVLTVLHQDWLNGKEYKCKVSNKGLPSSIEKTISKAKGQPREPQVYTLPPSQEEMTKNQVSLTCLVKGFYPSDIAVEWESNGQPENNYKTTPPVLDSDGSFFLYSRLTVDKSRWQEGNVFSCSVMHEALHNHYTQKSLSLSLGK